European Patent Specification EP 3 686 602 B1, published May 20, 2026. Title: MSP Nanopores and Related Methods. Applicant: University of Washington University of Alabama Research Foundation. The sequence listing filed with the application follows.

SEQUENCE LISTING (52 sequences)

SEQ ID NO: 1 - protein, 184 aa, Mycobacteria Smegmatis
GLDNELSLVDGQDRTLTVQQWDTFLNGVFPLDRNRLTREWFHSGRAKYIVAGPGADEFEGTLELGYQIGFPWSLGVGINFSYTTPNILIDDGDITAPPFGLNSVITPNLFPGVSISADLGNGPGIQEVATFSVDVSGAEGGVAVSNAHGTVTGAAGGVLLRPFARLIASTGDSVTTYGEPWNMN

SEQ ID NO: 2 - protein, 184 aa, Mycobacteria Smegmatis
GLDNELSLVDGQDRTLTVQQWDTFLNGVFPLDRNRLTREWFHSGRAKYIVAGPGADEFEGTLELGYQIGFPWSLGVGINFSYTTPNILIDDGDITAPPFGLNSVITPNLFPGVSISADLGNGPGIQEVATFSVDVSGPAGGVAVSNAHGTVTGAAGGVLLRPFARLIASTGDSVTTYGEPWNMN

SEQ ID NO: 3 - protein, 15 aa, Artificial Sequence
  Linker Peptide between MspA Peptides
GGGGSGGGGSGGGGS

SEQ ID NO: 4 - DNA, 72 bp, Artificial Sequence
  Oligonucleotides
gctgttgctctctcgcaacagcaaaaaaaaaaaaaaaaaaaaaaaaaaaaaaaaaaaaaaaaaaaaaaaaaa

SEQ ID NO: 5 - DNA, 76 bp, Artificial Sequence
  Oligonucleotides
gctctgttgctctctcgcaacagagcaaaaaaaaaaaaaaaaaaaaaaaaaaaaaaaaaaaaaaaaaaaaaaaaaa

SEQ ID NO: 6 - DNA, 80 bp, Artificial Sequence
  Oligonucleotides
gctgtctgttgctctctcgcaacagacagcaaaaaaaaaaaaaaaaaaaaaaaaaaaaaaaaaaaaaaaaaaaaaaaaaa

SEQ ID NO: 7 - DNA, 75 bp, Artificial Sequence
  Oligonucleotides
ccccccaaaaaaaaaaaaaaaaaaaaaaaaaaaaaaaaaaaaaaaaaaaaaaaaaaaaaactctattcttatctc

SEQ ID NO: 8 - DNA, 75 bp, Artificial Sequence
  Oligonucleotides
ccccccaaaaaaaaaaaaaaaaaaaaaaaaaaaaaaaaaaaaaaaaaaaaaaaaaaaaaacacacacacacacac

SEQ ID NO: 9 - DNA, 15 bp, Artificial Sequence
  Oligonucleotides
gagataagaatagag

SEQ ID NO: 10 - DNA, 50 bp, Artificial Sequence
  Oligonucleotides
aaaaaaaaaaaaaaaaaaaaaaaaaaaaaaaaaaaaaaaaaaaaaaaaaa

SEQ ID NO: 11 - DNA, 50 bp, Artificial Sequence
  Oligonucleotides
aaaaaaccccaaaaaaaaaaaaaaaaaaaaaaaaaaaaaaaaaaaaaaaa

SEQ ID NO: 12 - DNA, 50 bp, Artificial Sequence
  Oligonucleotides
aaaccccaaaaaaaaaaaaaaaaaaaaaaaaaaaaaaaaaaaaaaaaaaa

SEQ ID NO: 13 - DNA, 50 bp, Artificial Sequence
  Oligonucleotides
aacaaaaaaaaaaaaaaaaaaaaaaaaaaaaaaaaaaaaaaaaaaaaaaa

SEQ ID NO: 14 - DNA, 50 bp, Artificial Sequence
  Oligonucleotides
caaaaaaaaaaaaaaaaaaaaaaaaaaaaaaaaaaaaaaaaaaaaaaaaa

SEQ ID NO: 15 - DNA, 50 bp, Artificial Sequence
  Oligonucleotides
ccccaaaaaaaaaaaaaaaaaaaaaaaaaaaaaaaaaaaaaaaaaaaaaa

SEQ ID NO: 16 - DNA, 50 bp, Artificial Sequence
  Oligonucleotides
cccccccccccccccccccccccccccccccccccccccccccccccccc

SEQ ID NO: 17 - DNA, 50 bp, Artificial Sequence
  Oligonucleotides
tttttttttttttttttttttttttttttttttttttttttttttttttt

SEQ ID NO: 18 - DNA, 50 bp, Artificial Sequence
  Oligonucleotides
gggaaaaaaaaaaaaaaaaaaaaaaaaaaaaaaaaaaaaaaaaaaaaaaa

SEQ ID NO: 19 - DNA, 45 bp, Artificial Sequence
  Oligonucleotides
ggcggtggcggtagcggcggtggcggtagcggcggtggcggtagc

SEQ ID NO: 20 - DNA, 549 bp, Mycobacteria Smegmatis
ggcctggacaacgagctgagcctcgttgatggccaggaccgcaccctcaccgtgcagcagtgggacaccttcctcaatggtgtgttccccctggaccgcaaccgtcttacccgtgagtggttccactccggtcgcgccaagtacatcgtggccggccccggtgccgacgagttcgagggcacgctggaactcggctaccagatcggcttcccgtggtcgctgggtgtgggcatcaacttcagctacaccaccccgaacatcctgatcgacgacggtgacatcaccgctccgccgttcggcctgaactcggtcatcaccccgaacctgttccccggtgtgtcgatctcggcagatctgggcaacggccccggcatccaggaagtcgcaacgttctcggtcgacgtctccggcgccgagggtggcgtggccgtgtcgaacgcccacggcaccgtgaccggtgcggccggcggtgtgctgctgcgtccgttcgcccgcctgatcgcctcgaccggtgactcggtcaccacctacggcgaaccctggaacatg

SEQ ID NO: 21 - DNA, 549 bp, Mycobacteria Smegmatis
  Mutant MspA Gene
ggcctagacaatgagcttagccttgttgacggccaagaccgaaccctgaccctccagcaatgggatacctttctcaacggtgtattcccgctggatcgcaatcgtctaacccgcgagtggttccattccggccgcgctaagtatatcgtagccggacccggggccgatgagtttgagggaacgctcgaacttggctatcagataggctttccgtggtcgctaggtgtcggcattaactttagctataccacaccgaatatcctcatcgatgacggcgacataaccgcgccgcctttcggtctgaattcggtaatcacgccgaatctgtttcccggggtgtctatctcagcagacctggggaacggtcccggaatccaagaagtggcaactttctccgtcgatgtctcgggcgcggagggcggcgtagccgtctcgaatgcccatggcacggtgacaggtgcagccgggggtgtactgctacgtccattcgcgcgcctaatcgcgtcgacaggtgattcggttaccacatacggtgaaccatggaatatg

SEQ ID NO: 22 - DNA, 549 bp, Mycobacteria Smegmatis
  Mutant MspA Gene
ggactggataacgaactgagtctggtagatgttcaggatcgcaatctcacagtgcaacagtgggacactttcctgaatggcgtgtttcccctcgaccggaaccgacttacgcgtgaatggtttcactcaggtcgtgccaaatacattgtggcgggcccgggtgcggacgaattcgaaggcaccctggagctcgggtaccaaatcggtttcccttggtccctgggcgtgggtatcaatttcagttacacgacccccaacattctgatagacgatggtgatatcacggctcccccgtttggcctcaactccgtcataacccccaacctcttccctggtgtctcgatttcggccgatctcggcaatggccctggcattcaggaggtcgctacgttttcggtggacgtgtccggtgccgaaggtggtgtggcggtgtccaacgcgcacggtaccgtcaccggcgcggcgggcggcgtgctcctgcggccgtttgcccggctgattgcctccaccggggactccgtcacgacctatggcgagccctggaacatg

SEQ ID NO: 23 - DNA, 549 bp, Mycobacteria Smegmatis
  Mutant MspA Gene
ggccttgacaacgagctaagcctagttgacggccaggaccgtaccctaaccctacagcagtgggatacctttctcaatagcgtcttcccactggaccgcaatcgtctgacccgagagtggttccactccgggcgcgcaaagtatatcgtcgccggtcccggtgccgacgagttcgagttcacgcttgaactaggctaccagattggcttcccgtggtcgcttggtgttggcataaacttcagctacaccactccgaacatcctaatcgacgacggggacattaccgcaccgccattcgggctgaactcggtgatcacaccgaacctgtttcccggagtgtcaatctccgcagatcagggtaacggacccgggatccaggaagttgcaaccttctcagtcgacgtctcaggcgcagaggggggcgtcgccgtatcgaacgcccacggcactgtgacgggtgccgccggtggtgtcctgctccgtcccttcgcacgcctcatcgcatcgacgggtgactcggtaaccacgtacggggaaccgtggaacatg

SEQ ID NO: 24 - DNA, 549 bp, Mycobacteria Smegmatis
  Mutant MspA Gene
gggctggataacgaactgagtctcctggatggacaggatcgcaatctcacggtgcagcagtgggacacattccttaatggggtgttcccccttgaccgtaaccggcttacacgtgaatggttccactcgggtcgggccaagtacatagtggctggccctggtgctgacgagttcgaaggcacactggaactcggttaccaaatcgggttcccctggtcactgggggtgggaatcaacttcagctacacaacccctaacatactgatagacgacggtgacatcactgctcctccgtttggccttaactcagtcattacccctaacctattccccggtgtttcgatatcggcggatcttggcaacggcccgggcatacaggaagtcgcgacgttctcggttgacgtttccggggccgagggtggggtggcagtgtcaaacgctcacgggaccgttaccggggcggcaggcggggtgcttctgcgcccgttcgcccgtctgatagcctcaaccggcgactcagtcacaacctacggcgagccctggaacatg

SEQ ID NO: 25 - DNA, 549 bp, Mycobacteria Smegmatis
  Mutant MspA Gene
ggactcgataatgaactcagtctagtagacggtcaagatcggaatctgacagtccaacaatgggatacttttctgaacggcgtctttccgctcgatcggaatcgactcacgcgcgaatggtttcattcagggcgtgcgaaatatattgtcgcggggccgggcgcggatgaatttgaaggtaccctcgagctggggtatcaaattggttttccttggtcccttggcgtcggtattaattttagttatacgacgcccaatattctcatagatgatggcgatataacggcgcccccatttgggctcaattccgtgataacgcccaatctctttcctggcgtctccatttccgccgacctcggtaatggtcctggtattcaagaggtggctaccttttccgtggatgtgtcgggtgcggaaggcggtgtagcggtatccaatgcgcatggtacagtcacaggcgccgcgggtggcgtcctcctccggccatttgcacggctaattgcgtccacgggggattccgtgacgacgtatggtcagccgtggaacatg

SEQ ID NO: 26 - DNA, 549 bp, Mycobacteria Smegmatis
  Mutant MspA Gene
gggctagataatcagcttagtcttgtggacgggcaagatcgaacgctgacgctccaacaatgggatacgtttctaaacggcgtatttccgctcgatcggaatcgactaacgcgcgaatggtttcattcgggccgagctaaatatatagtagcaggaccgggggcagatgaatttgaaggaacactcgagcttgggtatcaaataggttttccttggtccctaggagtcgggattaattttagttatacaacacccaatatactcattgatgatggcgatataacggcgcctccttttggtctcaattccgtaattacgcctaatctctttccgggggtgtctatatcagccgacctcgggaacggtccaggaattcaagaggtggcgactttttccgtggatgtttcgggagcggaaggcggtgtagcagcgtccaatgctcatggaacggtcacaggcgcagcaacaggagtactcccacggccatttgcgcggctaattgcgtctacaggcgattccgttacgacatatggtgagccatggaatatg

SEQ ID NO: 27 - DNA, 549 bp, Mycobacteria Smegmatis
  Mutant MspA Gene
ggacttgataacgaactaagtctggtagatggtcaggatcgtaatcttacagttcaacagtgggacactttcctgaatggcgtttttcctctcgaccggaaccgactgacgcgggaatggtttcactcaggccgtgcaaaatacaatgtagcgggtccgggagcggacgaattcgaagggaccctagagcttgggtaccaaatgggtttcccttggtccctcggcgtaggtataaatttcagttacacgacacccaacattcttatagacgatggggatattacggcacccccctttggtctcaactccgtaataacacccaacctcttccctggagtctctatttcagccgatctcggaaatggacctggaattcaggaggttgctacattttctgtggacgtgtcaggtgcagaaggaggtgtcgcggtctccaacgcgcacggtacggtcacgggcgctgcggggggcgttctccttcggccctttgcgcggctcattgcttccacaggggactccgtaacgacttatggacagccttggaatatg

SEQ ID NO: 28 - protein, 211 aa, Mycobacteria Smegmatis
  MspA Protein
MKAISRVLIAMVAAIAALFTSTGTSHAGLDNELSLVDGQDRTLTVQQWDTFLNGVFPLDRNRLTREWFHSGRAKYIVAGPGADEFEGTLELGYQIGFPWSLGVGINFSYTTPNILIDDGDITAPPFGLNSVITPNLFPGVSISADLGNGPGIQEVATFSVDVSGAEGGVAVSNAHGTVTGAAGGVLLRPFARLIASTGDSVTTYGEPWNMN

SEQ ID NO: 29 - protein, 215 aa, Mycobacteria Smegmatis
  MspB Protein
MTAFKRVLIAMISALLAGTTGMFVSAGAAHAGLDNELSLVDGQDRTLTVQQWDTFLNGVFPLDRNRLTREWFHSGRAKYIVAGPGADEFEGTLELGYQIGFPWSLGVGINFSYTTPNILIDDGDITAPPFGLNSVITPNLFPGVSISADLGNGPGIQEVATFSVDVSGPAGGVAVSNAHGTVTGAAGGVLLRPFARLIASTGDSVTTYGEPWNMN

SEQ ID NO: 30 - protein, 215 aa, Mycobacteria Smegmatis
  MspC Protein
MKAISRVLIAMISALAAAVAGLFVSAGTSHAGLDNELSLVDGQDRTLTVQQWDTFLNGVFPLDRNRLTREWFHSGRAKYIVAGPGADEFEGTLELGYQIGFPWSLGVGINFSYTTPNILIDDGDITGPPFGLESVITPNLFPGVSISADLGNGPGIQEVATFSVDVSGPAGGVAVSNAHGTVTGAAGGVLLRPFARLIASTGDSVTTYGEPWNMN

SEQ ID NO: 31 - protein, 207 aa, Mycobacteria Smegmatis
  MspD Protein
MRYLVMMFALLVSVTLVSPRPANAVDNQLSVVDGQGRTLTVQQAETFLNGVFPLDRNRLTREWFHSGRATYHVAGPGADEFEGTLELGYQVGFPWSLGVGINFSYTTPNILIDGGDITQPPFGLDTIITPNLFPGVSISADLGNGPGIQEVATFSVDVKGAKGAVAVSNAHGTVTGAAGGVLLRPFARLIASTGDSVTTYGEPWNMN

SEQ ID NO: 32 - DNA, 50 bp, Artificial Sequence; identical to SEQ ID NO: 17
  Oligonucleotides

SEQ ID NO: 33 - DNA, 50 bp, Artificial Sequence
  Oligonucleotides
aaaaaaaaaaaaaaaaaaaaaaaaaaaaaaaaaaaaaaaaaaaaaaaaca

SEQ ID NO: 34 - DNA, 50 bp, Artificial Sequence
  Oligonucleotides
aaaaaaaaaaaaaaaaaaaaaaaaaaaaaaaaaaaaaaaaaaaaaaaaat

SEQ ID NO: 35 - DNA, 50 bp, Artificial Sequence
  Oligonucleotides
aaaaaaaaaaaaaaaaaaaaaaaaaaaaaaaaaaaaaaaaaaaaaaaata

SEQ ID NO: 36 - DNA, 50 bp, Artificial Sequence
  Oligonucleotides
aaaaaaaaaaaaaaaaaaaaaaaaaaaaaaaaaaaaaaaaaaaaaaataa

SEQ ID NO: 37 - DNA, 50 bp, Artificial Sequence
  Oligonucleotides
ccccccccccccccccccccccccccccccccccccccccccccccccca

SEQ ID NO: 38 - DNA, 50 bp, Artificial Sequence
  Oligonucleotides
ccccccccccccccccccccccccccccccccccccccccccccccccac

SEQ ID NO: 39 - DNA, 50 bp, Artificial Sequence
  Oligonucleotides
cccccccccccccccccccccccccccccccccccccccccccccccacc

SEQ ID NO: 40 - DNA, 58 bp, Artificial Sequence
  Oligonucleotides
cccccccccccccccccccccccccccccccccccccccccccccccccccccccccc

SEQ ID NO: 41 - DNA, 20 bp, Artificial Sequence
  Oligonucleotides
cgaccagcacggcatacatc

SEQ ID NO: 42 - DNA, 20 bp, Artificial Sequence
  Oligonucleotides
cgttctcggctcgatgatcc

SEQ ID NO: 43 - DNA, 27 bp, Artificial Sequence
  Oligonucleotides
cctgatcaacaacggtaacatcaccgc

SEQ ID NO: 44 - DNA, 21 bp, Artificial Sequence
  Oligonucleotides
ctgggcacgcctgggcaacgg

SEQ ID NO: 45 - DNA, 21 bp, Artificial Sequence
  Oligonucleotides
tccggcgcccgcggtggcgtg

SEQ ID NO: 46 - DNA, 19 bp, Artificial Sequence
  Oligonucleotides
ggcgccaagggtggcgtgg

SEQ ID NO: 47 - DNA, 20 bp, Artificial Sequence
  Oligonucleotides
cgttctcggtccgcgtctcc

SEQ ID NO: 48 - DNA, 50 bp, Artificial Sequence; identical to SEQ ID NO: 16
  Oligonucleotides

SEQ ID NO: 49 - DNA, 50 bp, Artificial Sequence; identical to SEQ ID NO: 10
  Oligonucleotides

SEQ ID NO: 50 - DNA, 52 bp, Artificial Sequence
  Oligonucleotides
aacccaaaaaaaaaaaaaaaaaaaaaaaaaaaaaaaaaaaaaaaaaaaaaaa

SEQ ID NO: 51 - DNA, 47 bp, Artificial Sequence
  Oligonucleotides
tacgcatacatcctaagaactcagactacctcccaataaatccacac

SEQ ID NO: 52 - DNA, 47 bp, Artificial Sequence
  Oligonucleotides
tcagactacctcccaataaatccgcagcaatcctcacacctaataat